European Patent Specification EP 3 305 807 B1, published August 21, 2024. Title: INTERACTION OF MORAXELLA CATARRHALIS WITH EPITHELIAL CELLS, EXTRACELLULAR MATRIX PROTEINS AND THE COMPLEMENT SYSTEM. Applicant: ARNE FORSGREN AB. The sequence listing filed with the application follows.

SEQUENCE LISTING (86 sequences)

SEQ ID NO: 1 - protein, 31 aa, Moraxella catarrhalis
DQKADIDNNINNIYELAQQQDQHSSDIKTLK

SEQ ID NO: 2 - protein, 154 aa, Moraxella catarrhalis
TGNGTVSVGKKGKERQIVHVGAGEISDTSTDAVNGSQLHVLATVVAQNKADIKDLDDEVGLLGEEINSLEGEIFNNQDAIAKNQADIKTLESNVEEGLLDLSGRLLDQKADIDNNINNIYELAQQQDQHSSDIKTLKNNVEEGLLDLSGRLIDQ

SEQ ID NO: 3 - protein, 154 aa, Moraxella catarrhalis
KDAIAKNNESIEDLYDFGHEVAESIGEIHAHNEAQNETLKGLITNSIENTNNITKNKADIQALENNVVEELFNLSGRLIDQKADIDNNINNIYELAQQQDQHSSDIKTLKKNVEEGLLELSDHIIDQKTDIAQNQANIQDLATYNELQDQYAQK

SEQ ID NO: 4 - protein, 721 aa, Moraxella catarrhalis
KVGKATNKISGGDNNTANGTYLTIGGGDYNKTKGRYSTIGGGLFNEATNEYSTIGSGGYNKAKGRYSTIGGGGYNEATNQYSTIGGGDNNTAKGRYSTIGGGGYNEATIENSTVGGGGYNQAKGRNSTVAGGYNNEATGTDSTIAGGRKNQATGKGSFAAGIDNKANADNAVALGNKNTIEGENSVAIGSNNTVKKGQQNVFILGSNTDTTNAQNGSVLLGHNTAGKAATIVNSAEVGGLSLTGFAGASKTGNGTVSVGKKGKERQIVHVGAGEISDTSTDAVNGSQLHVLATVVAQNKADIKDLDDEVGLLGEEINSLEGEIFNNQDAIAKNQADIKTLESNVEEGLLDLSGRLLDQKADIDNNINNIYELAQQQDQHSSDIKTLKNNVEEGLLDLSGRLIDQKADLTKDIKALESNVEEGLLDLSGRLIDQKADIAKNQADIAQNQTDIQDLAAYNELQDAYAKQQTEAIDALNKASSANTDRIATAELGIAENKKDAQIAKAQANENKDGIAKNQADIQLHDKKITNLGILHSMVARAVGNNTQGVATNKADIAKNQADIANNIKNIYELAQQQDQHSSDIKTLAKVSAANTDRIAKNKAEADASFETLTKNQNTLIEQGEALVEQNKAINQELEGFAAHADVQDKQILQNQADITTNKTAIEQNINRTVANGFEIEKNKAGIATNKQELILQNDRLNRINETNNHQDQKIDQLGYAL

SEQ ID NO: 5 - protein, 443 aa, Moraxella catarrhalis
KVGKATNKISGGDNNTANGTYLTIGGGDYNKTKGRYSTIGGGLFNEATNEYSTIGSGGYNKAKGRYSTIGGGGYNEATNQYSTIGGGDNNTAKGRYSTIGGGGYNEATIENSTVGGGGYNQAKGRNSTVAGGYNNEATGTDSTIAGGRKNQATGKGSFAAGIDNKANADNAVALGNKNTIEGENSVAIGSNNTVKKGQQNVFILGSNTDTTNAQNGSVLLGHNTAGKAATIVNSAEVGGLSLTGFAGASKTGNGTVSVGKKGKERQIVHVGAGEISDTSTDAVNGSQLHVLATVVAQNKADIKDLDDEVGLLGEEINSLEGEIFNNQDAIAKNQADIKTLESNVEEGLLDLSGRLLDQKADIDNNINNIYELAQQQDQHSSDIKTLKNNVEEGLLDLSGRLIDQKADLTKDIKALESNVEEGLLDLSGRLIDQKADIAKNQAD

SEQ ID NO: 6 - protein, 510 aa, Moraxella catarrhalis
QAKNDITLEDLPYLIKKIDQNELEADIGDITALEKYLALSQYGNILALEELNKALEELDEDVGWNQNDIANLEDDVETLTKNQNAFAEQGEAIKEDLQGLADFVEGQEGKILQNETSIKKNTQRNLVNGFEIEKNKDAIAKNNESIEDLYDFGHEVAESIGEIHAHNEAQNETLKGLITNSIENTNNITKNKADIQALENNVVEELFNLSGRLIDQKADIDNNINNIYELAQQQDQHSSDIKTLKKNVEEGLLELSDHIIDQKTDIAQNQANIQDLATYNELQDQYAQKQTEAIDALNKASSENTQNIEDLAAYNELQDAYAKQQTEAIDALNKASSENTQNIEDLAAYNELQDAYAKQQAEAIDALNKASSENTQNIAKNQADIANNITNIYELAQQQDKHRSDIKTLAKTSAANTDRIAKNKADDDASFETLTKNQNTLIEKDKEHDKLITANKTAIDANKASADTKFAATADAFTKNGNAITKNAKSITDLGTKVDGFDSRVTALDT

SEQ ID NO: 7 - protein, 322 aa, Moraxella catarrhalis
QAKNDITLEDLPYLIKKIDQNELEADIGDITALEKYLALSQYGNILALEELNKALEELDEDVGWNQNDIANLEDDVETLTKNQNAFAEQGEAIKEDLQGLADFVEGQEGKILQNETSIKKNTQRNLVNGFEIEKNKDAIAKNNESIEDLYDFGHEVAESIGEIHAHNEAQNETLKGLITNSIENTNNITKNKADIQALENNVVEELFNLSGRLIDQKADIDNNINNIYELAQQQDQHSSDIKTLKKNVEEGLLELSDHIIDQKTDIAQNQANIQDLATYNELQDQYAQKQTEAIDALNKASSENTQNIEDLAAYNELQDAYA

SEQ ID NO: 8 - protein, 148 aa, Moraxella catarrhalis
QAKNDITLEDLPYLIKKIDQNELEADIGDITALEKYLALSQYGNILALEELNKALEELDEDVGWNQNDIANLEDDVETLTKNQNAFAEQGEAIKEDLQGLADFVEGQEGKILQNETSIKKNTQRNLVNGFEIEKNKDAIAKNNESIED

SEQ ID NO: 9 - protein, 340 aa, Moraxella catarrhalis
NETLKGLITNSIENTNNITKNKADIQALENNVVEELFNLSGRLIDQKADIDNNINNIYELAQQQDQHSSDIKTLKKNVEEGLLELSDHIIDQKTDIAQNQANIQDLATYNELQDQYAQKQTEAIDALNKASSENTQNIEDLAAYNELQDAYAKQQTEAIDALNKASSENTQNIEDLAAYNELQDAYAKQQAEAIDALNKASSENTQNIAKNQADIANNITNIYELAQQQDKHRSDIKTLAKTSAANTDRIAKNKADDDASFETLTKNQNTLIEKDKEHDKLITANKTAIDANKASADTKFAATADAFTKNGNAITKNAKSITDLGTKVDGFDSRVTALDT

SEQ ID NO: 10 - protein, 157 aa, Moraxella catarrhalis
IQDLATYNELQDQYAQKQTEAIDALNKASSENTQNIEDLAAYNELQDAYAKQQTEAIDALNKASSENTQNIEDLAAYNELQDAYAKQQAEAIDALNKASSENTQNIAKNQADIANNITNIYELAQQQDKHRSDIKTLAKTSAANTDRIAKNKADDDA

SEQ ID NO: 11 - protein, 922 aa, Moraxella catarrhalis
MNKIYKVKKNAAGHLVACSEFAKGHTKKAVLGSLLIVGILGMATTASAQKAANTTNQASGRHTYVGGGDNNQATGMYSFIGGGFFNQATGNHLTIGGGSANQAKGNYSTIGGGDGNETTGTHSTIGGGDSNKAEGTHSTIGGGYDNTAKGTHSTIVGGRKNRAEGNYSTVAGGDNNQATGNNSTVVGGSKNQATGAGSFAAGVENQAKTENAVALGNKNTIGGTNSVAIGSNNTVEDGKQDVFILGSNTTNAQSGSVLLGNNTSGKAATAVSSATVGRLKLTGFAGVSQANQANSGTVSVGSAGSERQIVNVGAGQISATSTDAVNGSQLHALATAVSQNQDNILTNRVDIQELKRKQENDIKEVVEMQNAIAEQADINKNHIQDLAKAQLAGVAVMEELDKHVEDLYEATNENLDKISQLDGAVFNNTQNIEDLAAYNELQDAYAKQQTEAIDALNKASSENTQNIAKNSNHIKTLESNVEEELLNLSGRLIDQKADIDNNINHIYELAQQQDQHSSDIKTLKNNVEEGLLDLSGRLIDQKADIAKNQADIAQNQTDIQDLAAYNELQDAYAKQQTEAIDALNKASSANTDRIATAELGIAENKKDAQIAKAQANENKDGIAKNQADIQLHDKKITNLGILHSMVARAVGNNTQGVATNKADIAKNQADIANNIKNIYELAQQQDQHSSDIKTLAKVSAANTDRIAKNKAEADASFETLTKNQNTLIEQGEALVEQNKAINQELEGFAAHADVQDKQILQNQADITTNKTAIEQNINRTVANGFEIEKNKAGIATNKQELILQNDRLNRINETNNHQDQKIDQLGYALKEQGQHFNNRISAVERQTAGGIANAIAIATLPSPSRAGEHHVLFGSGYHNGQAAVSLGAAGLSDTGKSTYKIGLSWSDAGGLSGGVGGSYRWK

SEQ ID NO: 12 - protein, 913 aa, Moraxella catarrhalis
MNKIYKVKKNAAGHLVACSEFAKGHTKKAVLGSLLIVGILGMATTASAQAINTGQGTVVDQNGNEAIGNYSTASGGDYNQAKGNYSTASGGSGNTAEGNYSTASGGLGNTAEGNYSTASGGLGNTAKGKYSTVAGGANNQAKGDYSTASGGSGNTAEGNYSTVAGGKNNQATGLNSTVAGGSDNQATGTGSFAAGVGNKANAENAVALGNKNTIEGENSVAIGSNNTVETGKENVFILGSGTTGVTSNSVLLGNKTAGKEATAVNDATVNGLTLKNFAGVSKTGNGTVSVGSENHERQIVNVGAGKISADSTDAVNGSQLHALATVVAKNKSDITKNQAETLVNRVNIKELERKQENDIKEVVEMQNAIAEQADKNKNHIQDLAKAQLAGVTVMEELNKHVEDLYEATNDNLDKISQLDGAVFNNTQNIAKNSNHIKTLENNVEEELLNLSGRLLDQKADIDNNINNIYELAQQQDQHSSDIKTLKNNVEEGLLDLSGRLIDQKADLTKDIKALENNVEEGLLDLSGRLIDQKADIAKNQADIAQNQTDIQDLAAYNELQDAYAKQQTEAIDALNKASSANTDRIATAELGIAENKKDAQIAKAQANENKDGIAKNQADIQLHDKKITNLGILHSMVARAVGNNTQGVATNKADIAKNQADIANNIKNIYELAQQQDQHSSDIKTLAKVSAANTDRIAKNKAEADASFETLTKNQNTLIEQGEALVEQNKAINQELEGFAAHADVQDKQILQNQADITTNKTAIEQNINRTVANGFEIEKNKAGIATNKQELILQNDRLNRINETNNRQDQKIDQLGYALKEQGQHFNNRISAVERQTAGGIANAIAIATLPSPSRAGEHHVLFGSGYHNGQAAVSLGAAGLSDTGKSTYKIGLSWSDAGGLSGGVGGSYRWK

SEQ ID NO: 13 - protein, 863 aa, Moraxella catarrhalis
MNKIYKVKKNAAGHLVACSEFAKGHTKKAVLGSLLIVGILGMATTASAQKVGKATNKISGGDNNTANGTYLTIGGGDYNKTKGRYSTIGGGLFNEATNEYSTIGSGGYNKAKGRYSTIGGGGYNEATNQYSTIGGGDNNTAKGRYSTIGGGGYNEATIENSTVGGGGYNQAKGRNSTVAGGYNNEATGTDSTIAGGRKNQATGKGSFAAGIDNKANADNAVALGNKNTIEGENSVAIGSNNTVKKGQQNVFILGSNTDTTNAQNGSVLLGHNTAGKAATIVNSAEVGGLSLTGFAGASKTGNGTVSVGKKGKERQIVHVGAGEISDTSTDAVNGSQLHALATVVAQNKADIKDLDDEVGLLGEEINSLEGEIFNNQDAIAKNQADIKTLESNVEEGLLDLSGRLLDQKADIDNNINNIYELAQQQDQHSSDIKTLKNNVEEGLLDLSGRLIDQKADLTKDIKALESNVEEGLLDLSGRLIDQKADIAKNQADIAQNQTDIQDLAAYNELQDAYAKQQTEAIDALNKASSANTDRIATAELGIAENKKDAQIAKAQANENKDGIAKNQADIQLHDKKITNLGILHSMVARAVGNNTQGVATNKADIAKNQADIANNIKNIYELAQQQDQHSSDIKTLAKVSAANTDRIAKNKAEADASFETLTKNQNTLIEQGEALVEQNKAINQELEGFAAHADVQDKQILQNQADITTNKTAIEQNINRTVANGFEIEKNKAGIATNKQELILQNDRLNRINETNNHQDQKIDQLGYALKEQGQHFNNRISAVERQTAGGIANAIAIATLPSPSRAGEHHVLFGSGYHNGQAAVSLGAAGLSDTGKSTYKIGLSWSDAGGLSGGVGGSYRWK

SEQ ID NO: 14 - protein, 892 aa, Moraxella catarrhalis
MNKIYKVKKNAAGHLVACSEFAKGHTKKAVLGSLLIVGALGMATTASAQATKGTGKHVVDNKDNKAKGDYSTASGGKDNEAKGNYSTVGGGDYNEAKGNYSTVGGGSSNTAKGEKSTIGGGDTNDANGTYSTIGGGYYSRAIGDSSTIGGGYYNQATGEKSTVAGGRNNQATGNNSTVAGGSYNQATGNNSTVAGGSHNQATGEGSFAAGVENKANANNAVALGKNNTIDGDNSVAIGSNNTIDSGKQNVFILGSSTNTTNAQSGSVLLGHNTAGKKATAVSSAKVNGLTLGNFAGASKTGNGTVSVGSENNERQIVNVGAGNISADSTDAVNGSQLYALATAVKADADENFKALTKTQNTLIEQGEAQDALIAQNQTDITANKTAIERNFNRTVVNGFEIEKNKAGIAKNQADIQTLENNVGEELLNLSGRLLDQKADIDNNINNIYDLAQQQDQHSSDIKTLKKNVEEGLLDLSGRLIDQKADLTKDIKTLENNVEEGLLDLSGRLIDQKADIAKNQADIAQNQTDIQDLAAYNELQDQYAQKQTEAIDALNKASSANTDRIATAELGIAENKKDAQIAKAQANENKDGIAKNQADIQLHDKKITNLGILHSMVARAVGNNTQGVATNKADIAKNQADIANNIKNIYELAQQQDQHSSDIKTLAKVSAANTDRIAKNKAEADASFETLTKNQNTLIEQGEALVEQNKAINQELEGFAAHADVQDKQILQNQADITTNKAAIEQNINRTVANGFEIEKNKAGIATNKQELILQNDRLNQINETNNRQDQKIDQLGYALKEQGQHFNNRISAVERQTAGGIANAIAIATLPSPSRAGEHHVLFGSGYHNGQAAVSLGAAGLSDTGKSTYKIGLSWSDAGGLSGGVGGSYRWK

SEQ ID NO: 15 - protein, 873 aa, Moraxella catarrhalis
MNKIYKVKKNAAGHLVACSEFAKGHTKKAVLGSLLIVGILGMATTASAQQTIARQGKGMHSIIGGGNDNEANGDYSTVSGGDYNEAKGDSSTIGGGYYNEANGDSSTIGGGFYNEAKGESSTIGGGDNNSATGMYSTIGGGDNNSATGRYSTIAGGWLNQATGHSSTVAGGWLNQATNENSTVGGGRFNQATGRNSTVAGGYKNKATGVDSTIAGGRNNQANGIGSFAAGIDNQANANNTVALGNKNIIKGKDSVAIGSNNTVETGKENVFILGSNTKDAHSNSVLLGNETTGKAATTVENAKVGGLSLTGFVGASKANTNNGTVSVGKQGKERQIVNVGAGQIRADSTDAVNGSQLHALATAVDAEFRTLTQTQNALIEQGEAINQELEGLADYTNAQDEKILKNQTDITANKTAIEQNFNRTVTNGFEIEKNKAGIAKNQADIQTLENDVGKELLNLSGRLLDQKADIDNNINNIYELAQQQDQHSSDIKTLKNNVEEGLLDLSGRLIDQKADLTKDIKALENNVEEGLLDLSGRLIDQKADIAKNQADIQDLAAYNELQDQYAQKQTEAIDALNKASSANTDRIATAELGIAENKKDAQIAKAQANENKDGIAKNQADIANNIKNIYELAQQQDQHSSDIKTLAKVSAANTDRIAKNKAEADASFETLTKNQNTLIEQGEALVEQNKAINQELEGFAAHADVQDKQILQNQADITANKTAIEQNINRTVANGFEIEKNKAGIATNKQELILQHDRLNRINETNNRQDQKIDQLGYALKEQGQHFNNRISAVERQTAGGIANAIAIATLPSPSRAGEHHVLFGSGYHNGQAAVSLGAAGLSDTGKSTYKIGLSWSDAGGLSGGVGGSYRWK

SEQ ID NO: 16 - protein, 832 aa, Moraxella catarrhalis
MNKIYKVKKNAAGHLVACSEFAKGHTKKAVLGSLLIVGALGMATTASAQATNSKGTGAHIGVNNNNEAPGDYSFIGSGGYNKAEGRYSAIGGGLFNKATNEYSTIVGGGYNKAEGRYSTIGGGSNNEATNEYSTIVGGDDNKATGRYSTIGGGDNNTAEGEYSTVAGGKNNQATGTGSFAAGVENQANAENAVAVGKKNIIEGENSVAIGSENTVKTEHKNVFILGSGTTGVTSNSVLLGNETAGKQATTVKNAEVGGLSLTGFAGESKAENGVVSVGSEGGERQIVNVGAGQISDTSTDAVNGSQLHALATVVDDNQYDIVNNRADILNNQDDIKDLQKEVKGLDNEVGELSRDINSLHDVTDNQQDDIKELKRGVKELDNEVGVLSRDINSLHDDVADNQDDIAKNKADIKGLNKEVKELDKEVGVLSRDIGSLHDDVATNQADIAKNQADIKTLENNVEEELLNLSGRLLDQKADIDNNINNIYELAQQQDQHSSDIKTLKNNVEEGLLDLSGRLIDQKADIAKNQADIAQNQTDIQDLAAYNELQDQYAQKQTEAIDALNKASSENTQNIAKNQADIANNINNIYELAQQQDQHSSDIKTLAKVSAANTDRIAKNKAEADASFETLTKNQNTLIEQGEALVEQNKAINQELEGFAAHADIQDKQILQNQADITTNKTAIEQNINRTVANGFEIEKNKAGIATNKQELILQNDRLNRINETNNRQDQKIDQLGYALKEQGQHFNNRISAVERQTAGGIANAIAIATLPSPSRAGEHHVLFGSGYHNGQAAVSLGAAGLSDTGKSTYKIGLSWSDAGGLSGGVGGSYRWK

SEQ ID NO: 17 - protein, 941 aa, Moraxella catarrhalis
MNKIYKVKKNAAGHLVACSEFAKGHTKKAVLGSLLIVGILGMATTASAQMATTPSAQVVKTNNKKNGTHPFIGGGDYNTTKGNYPTIGGGHFNTAEGNYSTVGGGFTNEAIGKNSTVGGGFTNEAMGEYSTVAGGANNQAKGNYSTVGGGNGNKAIGNNSTVVGGSNNQAKGEHSTIAGGKNNQATGNGSFAAGVENKADANNAVALGNKNTIEGTNSVAIGSNNTVKTGKENVFILGSNTNTENAQSGSVLLGNNTAGKAATTVNNAEVNGLTLENFAGASKANANNIGTVSVGSENNERQIVNVGAGQISATSTDAVNGSQLHALAKAVAKNKSDIKGLNKGVKELDKEVGVLSRDINSLHDDVADNQDSIAKNKADIKGLNKEVKELDKEVGVLSRDIGSLHDDVADNQDSIAKNKADIKGLNKEVKELDKEVGVLSRDIGSLHDDVATNQADIAKNQADIKTLENNVEEELLNLSGRLIDQKADIDNNINNIYELAQQQDQHSSDIKTLKNNVEEGLLDLSGRLIDQKADLTKDIKTLKNNVEEGLLDLSGRLIDQKADIAKNQADIAQNQTDIQDLAAYNELQDQYAQKQTEAIDALNKASSANTDRIATAELGIAENKKDAQIAKAQANENKDGIAKNQADIQLHDKKITNLGILHSMVARAVGNNTQGVATNKADIAKNQADIANNIKNIYELAQQQDQHSSDIKTLAKVSAANTDRIAKNKAEADASFETLTKNQNTLIEQGEALVEQNKAINQELEGFAAHADVQDKQILQNQADITTNKTAIEQNINRTVANGFEIEKNKAGIATNKQELILQNDRLNQINETNNHQDQKIDQLGYALKEQGQHFNNRISAVERQTAGGIANAIAIATLPSPSRAGEHHVLFGSGYHNGQAAVSLGAAGLSDTGKSTYKIGLSWSDAGGLSGGVGGSYRWK

SEQ ID NO: 18 - protein, 912 aa, Moraxella catarrhalis
MNKIYKVKKNAAGHLVACSEFAKGHTKKAVLGSLLIVGILGMATTASAQQNNQKSGKYPFIGGGGYNNVDGKYPTIGGGLFNIANGKYPTIGGGAHNKANGTYSTIGGGSYNEANGEKSTIGGGDNNTAKGNHSTVVGGYKNEATGKYSTVGGGNSNKAEGTDSTIAGGKNNQAKGEGSFAAGVENKANAENAVAVGKKNSIEGKDSVAIGSENTVENNKQNVFILGSKTSGAQSNSVLLGNETTGKAATTVENAEVGGLSLTGFAGASKANANANIGTVSVGSQGKERQIVNVGAGQISATSTDAVNGSQLHALASTIDEEVDLLGEEINSLEGEIFNNQDAIAKNQADIATNKTNIETNGSKITNLGTLYATVTKAVGNNTQGVAANKADITKNKADIQDLDDEVGVLSQDIGSLHDDVATNQADIAKNQADIQTLENNVEEELLNLSGRLLDQKADIDNNINNIYELAQQQDQHSSDIKTLKNNVEEGLLDLSGRLIDQKADLTKDIKTLESNVEEGLLDLSGRLIDQKADIAKNQADIAQNQTDIQDLAAYNELQDQYAQKQTEAIDALNKASSANTDRIATAELGIAENKKDAQIAKAQANENKDGIAKNQADIQLHDKKITNLGILHSMVARAVGNNTQGVATNKADIAKNQADIANNIKNIYELAQQQDQHSSDIKTLAKVSAANTDRIAKNKAEADASFETLTKNQNTLIEQGEALVEQNKAINQELEGFAAHADVQDKQILQNQADITTNKTAIEQNINRTVANGFEIEKNKAGIATNKQELILQNDRLNRINETNNHQDQKIDQLGYALKEQGQHFNNRISAVERQTAGGIANAIAIATLPSPSRAGEHHVLFGSGYHNGQAAVSLGAAGLSDTGKSTYKIGLSWSDAGGLSGGVGGSYRWK

SEQ ID NO: 19 - protein, 877 aa, Moraxella catarrhalis
MNKIYKVKKNAAGHSVACSEFAKGHTKKAVLGSLLIVGALGMATTASAQLVSTTQPNDYRSSTTGNNHLGSSWSIIGAGHDNIVYRSASNSGILSGYKNRVNGSTSAIVGGYDNETRGKYTFVGGGYKNLAEGHQSAIGGGYANWAEGDNATIAGGFENFAAGNQSAIGGGYANLAEGDDATIAGGFENRAEGNQSAIGGGYANFAAGDYTFVGGGYENRAEGNQSAIGGGYANLAEGDNATIAGGFENRAKGINSVVSGGYANQATGESSTIAGGFENRAEGIDSVVSGGYANQANGAQSTVAGGYNNQATGESSTIAGGSNNQATGTGSFAAGVENKANADNAVALGKNNIINGDNSAAIGSNNTVKKGQKDVFILGSNTSGAQSNSVLLGNETTGKKATAVENATVGDLSLTGFAGVSKANSGTVSVGSEGKERQIVHVGAGRISNDSTDAVNGSQLYALAAAVDDNQYDIEKNQDDIKELKRGVKELDKEMNVLSRDIVSLNDDVAQNQSDIKTLKNNVEEGLLELSGHLIDQKADLTKDIKALENNVEEGLLDLSGRLLDQKADIAKNQADIAQNQTDIQDLAAYNELQDAYAKQQTEAIDALNKASSENTQNIEDLAAYNELQDAYAKQQTEAIDALNKASSENTQNIAKNQADIANNINNIYELAQQQDQHSSDIKTLAKASAANTDRIAKNKADADASFETLTKNQNTLIEKDKEHDKLITANKTAIDANKASADTKFAATADAITKNGNAITKNAKSITDLGTKVDGFDGRVTALDTKVNAFDGRITALDSKVENGMAAQAALSGLFQPYSVGKFNATAALGGYGSKSAVAIGAGYRVNPNLAFKAGAAINTSGNKKGSYNIGVNYEF

SEQ ID NO: 20 - protein, 889 aa, Moraxella catarrhalis
MNKIYKVKKNAAGHLVACSEFAKGHTKKAVLGSLLIVGALGMATTASAQPLVSTNKPNQQVKGYWSIIGAGRHNNVGGSAHHSGILGGWKNTVNGYTSAIVGGYGNETQGDYTFVGGGYKNLAKGNYTFVGGGYKNLAEGDNATIAGGFANLAEGDNATIAGGFENRAEGIDSVVSGGYANQATGESSTVAGGSNNLAEGKSSAIGGGRQNEASGDRSTVSGGYNNLAEGKSSAIGGGEFNLALGNNATISGGRQNEASGDRSTVAGGEQNQAIGKYSTISGGRQNEASGDRSTVAGGEQNQAIGKYSTVSGGYRNQATGKGSFAAGIDNKANADNAVALGNKNTIEGENSVAIGSNNTVKKNQKNVFILGSNTDTKDAQSGSVLLGDNTSGKAATAVEDATVGDLSLTGFAGVSKANSGTVSVGSEGKERQIVHVGAGRISNDSTDAVNGSQLYALAAAVDDNQYDIEKNQDDIAKNQADIAKNQADIQTLENDVGKELLNLSGRLIDQKADIDNNINHIYELAQQQDQHSSDIKTLKKNVEEGLLELSGHLIDQKADLTKDIKALESNVEEGLLDLSGRLIDQKADIAQNQANIQDLAAYNELQDQYAQKQTEAIDALNKASSENTQNIEDLAAYNELQDAYAKQQTEAIDALNKASSENTQNIAKNQADIANNINNIYELAQQQDQHSSDIKTLAKASAANTDRIAKNKADADASFETLTKNQNTLIEKDKEHDKLITANKTAIDANKASADTKFAATADAITKNGNAITKNAKSITDLGTKVDGFDGRVTALDTKVNAFDGRITALDSKVENGMAAQAALSGLFQPYSVGKFNATAALGGYGSKSAVAIGAGYRVNPNLAFKAGAAINTSGNKKGSYNIGVNYEF

SEQ ID NO: 21 - protein, 686 aa, Moraxella catarrhalis
MKTMKLLPLKIAVTSAMIIGLGAASTANAQATETFLPNLFDNDYTETTDPLYHGMILGNTAITQDTQYKFYAENGNEVPDSLFFNKILHDQQLNGFKEGDTIIPLDENGKPVYKLDEITENGVKRKVYSVTTKTATREDVEQSAYSRGIQGDIDDLYEANKENVNRLIEHGDKIFANEESVQYLNKEVQNNIENIHELAQQQDQHSSDIKTLKKNVEEGLLELSGRLIAQKEDIAQNQTDIQDLATYNELQDQYAQKQTEAIDALNKASSENTQNIAKNSNHIKTLENNIEEGLLELSGHLIDQKADLTKDIKALESNVEEGLLDLSGRLLDQKADIAKNQADIAQNQTDIQDLAAYNELQDQYAQKQTEAIDALNKASSENTQNIEDLAAYNELQDAYAKQQTEAIDALNKASSENTQNIEDLAAYNELQDAYAKQQTEAIDALNKASSENTQNIAKNQADIANNINNIYELAQQQDQHSSDIKTLAKASAANTDRIAKNKADADASFETLTKNQNTLIEKDKEHDKLITANKTAIDANKASADTKFAATADAITKNGNAITKNAKSITDLGTKVDGFDGRVTALDTKVNALDTKVNAFDGRITALDSKVENGMAAQAALSGLFQPYSVGKFNATAALGGYGSKSAVAIGAGYRVNPNLAFKAGAAINTSGNKKGSYNIGVNYEF

SEQ ID NO: 22 - protein, 684 aa, Moraxella catarrhalis
MKTMKLLPLKIAVTSAMMVGLGMASTANAQQQKSPKTEIFLPNLFDNDNTELTDPLYHNMILGNTALLTQENQYKFYADDGNGVPDSLLFNKILHDQLLHGFKEGDTIIPLDENGKPVYKLDSIVEQGKTKTVYSVTTKTATADDVNSAYSRGIQGDIDDLYEANKENVNRLIEHGDKIFANEESVQYLNREVQNNIENIHELAQQQDQHSSDIKTLKKNVEKDLLDLSGRLIAQKEDIAQNQTDIQDLATYNELQDQYAQKQTEAIDALNKASSENTQNIAKNSNHIKTLENNIEEGLLELSGHLIDQKADLTKDIKALESNVEEGLLDLSGRLIDQKADIAQNQANIQDLAAYNELQDAYAKQQTEAIDALNKASSENTQNIEDLAAYNELQDAYAKQQTEAIDALNKASSENTQNIEDLAAYNELQDAYAKQQTEAIDALNKASSENTQNIAKNQADIANNINNIYELAQQQDQHSSDIKTLAKASAANTDRIAKNKADADASFETLTKNQNTLIEKDKEHDKLITANKTAIDANKASADTKFAATADAITKNGNAITKNAKSITDLGTKVDGFDGRVTALDTKVNALDTKVNAFDGRITALDSKVENGMAAQAALSGLFQPYSVGKFNATAALGGYGSKSAVAIGAGYRVNPNLAFKAGAAINTSGNKKGSYNIGVNYEF

SEQ ID NO: 23 - protein, 576 aa, Moraxella catarrhalis
MKTMKLLPLKIAVTSAMIVGLGATSTVNAQVVEQFFPNIFFNENHDELDDAYHNMILGDTAIVSNSQDNSTQLKFYSNDEDSVPDSLLFSKLLHEQQLNGFKAGDTIIPLDKDGKPVYTKDTRTKDGKVETVYSVTTKIATQDDVEQSAYSRGIQGDIDDLYDINREVNEYLKATHDYNERQTEAIDALNKASSANTDRIDTAEERIDKNEYDIKALESNVEEGLLELSGHLIDQKADLTKDIKALESNVEEGLLELSGHLIDQKADLTKDIKALESNVEEGLLDLSGRLLDQKADIAKNQADIAQNQTDIQDLAAYNELQDAYAKQQTEAIDALNKASSENTQNIAKNQADIANNINNIYELAQQQDQHSSDIKTLAKASAANTDRIAKNKADADASFETLTKNQNTLIEKDKEHDKLITANKTAIDANKASADTKFAATADAITKNGNAITKNAKSITDLGTKVDGFDGRVTALDTKVNALDTKVNAFDGRITALDSKVENGMAAQAALSGLFQPYSVGKFNATAALGGYGSKSAVAIGAGYRVNPNLAFKAGAAINTSGNKKGSYNIGVNYEF

SEQ ID NO: 24 - protein, 674 aa, Moraxella catarrhalis
MKTMKLLPLKIAVTSAMIVGLGATSTVNAQVVEQFFPNIFFNENHDELDDAYHNMILGDTAIVSNSQDNSTQLKFYSNDEDSVPDSLLFSKLLHEQQLNGFKAGDTIIPLDKDGKPVYTKDTRTKDGKVETVYSVTTKIATQDDVEQSAYSRGIQGDIDDLYDINREVNEYLKATHDYNERQTEAIDALNKASSANTDRIDTAEERIDKNEYDIKALESNVEEGLLELSGHLIDQKADLTKDIKALESNVEEGLLELSGHLIDQKADLTKDIKALESNVEEGLLDLSGRLIDQKADIAQNQANIQDLAAYNELQDAYAKQQTEAIDALNKASSENTQNIEDLAAYNELQDAYAKQQTEAIDALNKASSENTQNIEDLAAYNELQDAYAKQQTEAIDALNKASSENTQNIEDLAAYNELQDAYAKQQTEAIDALNKASSENTQNIAKNQADIANNINNIYELAQQQDQHSSDIKTLAKASAANTDRIAKNKADADASFETLTKNQNTLIEKDKEHDKLITANKTAIDANKASADTKFAATADAITKNGNAITKNAKSITDLGTKVDGFDGRVTALDTKVNALDTKVNAFDGRITALDSKVENGMAAQAALSGLFQPYSVGKFNATAALGGYGSKSAVAIGAGYRVNPNLAFKAGAAINTSGNKKGSYNIGVNYEF

SEQ ID NO: 25 - protein, 650 aa, Moraxella catarrhalis
MKTMKLLPLKIAVTSALIVGLGAASTANAQQQQKTKTEVFLPNLFYNDYIEETDLLYHNMILGDTAALVDRQNYSNSQLKFYSNDEESVPDSLLFSKMLNNQQLNGFKAGDIIIPVDANGQVIYQKDTRVEGGKTRTVLSVTTKIATQQDVDSAYSRGIQGKVNDLDDEMNFLNHDITSLYDVTANQQDDIKGLKKGVKDLKKGVKGLNKELKELDKEVGVLSRDIGSLNDDVAQNNESIEDLYDFSQEVADSIGEIHAHNKAQNETLQDLITNSVENTNNITKNKADIQALENNVVEELFNLSGRLIDQKADLTKDIKTLESNVEEGLLELSGHLIDQKADIAKNQADIAQNQANIQDLAAYNELQDAYAKQQTEAIDALNKASSENTQNIEDLAAYNELQDAYAKQQTEAIDALNKASSENTQNIAKNQADIANNINNIYELAQQQDQHSSDIKTLAKASAANTDRIAKNKADADASFETLTKNQNTLIEKDKEHDKLITANKTAIDENKASADTKFAATADAITKNGNAITKNAKSITDLGTKVDGFDGRVTALDTKVNAFDGRITALDSKVENGMAAQAALSGLFQPYSVGKFNATAALGGYGSKSAVAIGAGYRVNPNLAFKAGAAINTSGNKKGSYNIGVNYEF

SEQ ID NO: 26 - protein, 668 aa, Moraxella catarrhalis
MKTMKLLPLKIAVTSALIVGLGTASTANAQVASPANQKIQQKIKKVRKELRQDIKSLRNDIDSNTADIGSLNDDVADNQDDILDNQADIAKNQDDIEKNQADIKELDKEVGVLSREIGSLNDDIADNYTDIIDNYTDIIDNQANIAKNQDDIEKNQADIKELDKEVGVLSREIGSLNDDVADNQDDIAKNQADIQTLENNVEEGLLELSGHLLDQKADIDNNINNIYELAQQQDQHSSDIKTLKKNVEEGLLELSGHLIDQKTDIAQNQANIQDLATYNELQDQYAQEQTEAIDALNKASSENTQNIAKNSNRIKALESNVEEGLLELSGHLIDQKADLTKDIKALESNVEEGLLELSGHLIDQKADIAQNQANIQDLAAYNELQDQYAQKQTEAIDALNKASSENTQNIEDLAAYNELQDAYAKQQTEAIDALNKASSENTQNIAKNQADIANNINNIYELAQQQDQHSSDIKTLAKASAANTDRIAKNKADADASFETLTKNQNTLIEKDKEHDKLITANKTAIDANKVSADTKFAATADAITKNGNAITKNAKSITDLGTKVDAFDSRVTALDTKVNAFDGRITALDSKVENGMAAQAALSGLFQPYSVGKFNATAALGGYGSKSAVAIGAGYRVNPNLAFKAGAAINTSGNKKGSYNIGVNYEF

SEQ ID NO: 27 - protein, 894 aa, Moraxella catarrhalis
MNKIYKVKKNAAGHSVACSEFAKGHTKKAVLGSLLIVGALGMATTASAQTGSTNAANGNIISGVGAYVGGGVINQAKGNYPTVGGGFDNRATGNYSVISGGFDNQAKGEHSTIAGGESNQATGRNSTVAGGSNNQAVGTNSTVAGGSNNQAKGANSFAAGVGNQANTDNAVALGKNNTINGNNSAAIGSENTVNENQKNVFILGSNTTNAQSGSVLLGHETSGKEATAVSRARVNGLTLKNFSGVSKADNGTVSVGSQGKERQIVHVGAGQISDDSTDAVNGSQLYALATAVDDNQYDIEINQDNIKDLQKEVKGLDKEVGVLSRDIGSLHDDVADNQADIAKNKADIKELDKEMNVLSRDIVSLNDDVADNQADIAKNQADIKTLENNVEEGLLDLSGRLIDQKADIDNNINHIYELAQQQDQHSSDIKTLKKNVEEGLLELSGHLIDQKADIAQNQTDIQDLATYNELQDQYAQKQTEAIDALNKASSENTQNIEDLAAYNELQDAYAKQQTEAIDALNKASSENTQNIEDLAAYNELQDAYAKQQTEAIDALNKASSENTQNIEDLAAYNELQDAYAKQQTEAIDALNKASSENTQNIQDLAAYNELQDAYAKQQTEAIDALNKASSENTQNIQDLAAYNELQDAYAKQQTEAIDALNKASSENTQNIAKNQADIANNINNIYELAQQQDQHSSDIKTLAKASAANTDRIAKNKADADASFETLTKNQNTLIEKDKEHDKLITANKTAIDANKASADTKFAATADAITKNGNAITKNAKSITDLGTKVDGFDGRVTALDTKVNAFDGRITALDSKVENGMAAQAALSGLFQPYSVGKFNATAALGGYGSKSAVAIGAGYRVNPNLAFKAGAAINTSGNKKGSYNIGVNYEF

SEQ ID NO: 28 - protein, 630 aa, Moraxella catarrhalis
MKTMKLLPLKIAVTSAMIIGLGAASTANAQAKNDITLEDLPYLIKKIDQNELEADIGDITALEKYLALSQYGNILALEELNKALEELDEDVGWNQNDIANLEDDVETLTKNQNAFAEQGEAIKEDLQGLADFVEGQEGKILQNETSIKKNTQRNLVNGFEIEKNKDAIAKNNESIEDLYDFGHEVAESIGEIHAHNEAQNETLKGLITNSIENTNNITKNKADIQALENNVVEELFNLSGRLIDQKADIDNNINNIYELAQQQDQHSSDIKTLKKNVEEGLLELSDHIIDQKTDIAQNQANIQDLATYNELQDQYAQKQTEAIDALNKASSENTQNIEDLAAYNELQDAYAKQQTEAIDALNKASSENTQNIEDLAAYNELQDAYAKQQAEAIDALNKASSENTQNIAKNQADIANNITNIYELAQQQDKHRSDIKTLAKTSAANTDRIAKNKADDDASFETLTKNQNTLIEKDKEHDKLITANKTAIDANKASADTKFAATADAFTKNGNAITKNAKSITDLGTKVDGFDSRVTALDTKVNAFDGRITALDSKVENGMAAQAALSGLFQPYSVGKFNATAALGGYGSKSAVAIGAGYRVNPNLAFKAGAAINTSGNKKGSYNIGVNYEF

SEQ ID NO: 29 - protein, 630 aa, Moraxella catarrhalis
MKTMKLLPLKIAVTSAMIIGLGAASTANAQAKNDITLEDLPYLIKKIDQNELEADIGDITALEKYLALSQYGNILALEELNKALEELDEDVGWNQNDIANLEDDVETLTKNQNALAEQGEAIKEDLQGLADFVEGQEGKILQNETSIKKNTQRNLVNGFEIEKNKDAIAKNNESIEDLYDFGHEVAESIGEIHAHNEAQNETLKGLITNSIENTNNITKNKADIQALENNVVEELFNLSGRLIDQKADIDNNINNIYELAQQQDQHSSDIKTLKKNVEEGLLELSGHLIDQKTDIAQNQANIQDLATYNELQDQYAQKQTEAIDALNKASSENTQNIEDLAAYNELQDAYAKQQTEAIDALNKASSENTQNIEDLAAYNELQDAYAKQQTEAIDALNKASSENTQNIAKNQADIANNINNIYELAQQQDQHSSDIKTLAKASAANTDRIAKNKADADASFETLTKNQNTLIEKDKEHDKLITANKTAIDANKASADTKFAATADAITKNGNAITKNAKSITDLGTKVDGFDSRVTALDTKVNAFDGRITALDSKVENGMAAQAALSGLFQPYSVGKFNATAALGGYGSKSAVAIGAGYRVNPNLAFKAGAAINTSGNKKGSYNIGVNYEF

SEQ ID NO: 30 - protein, 616 aa, Moraxella catarrhalis
MKTMKLLPLKIAVTSALIVGLGAVSTTNAQAQSRSLDQIQTKLADLAGKIAAGKNGGGQNNQNNQNDINKYLFLSQYANILTMEELNNNVVKNSSSIETLETDFGWLENDVADLEDGVEELTKNQNTLIEKDEEHDRLIAQNQADIQTLENNVVEELFNLSDRLIDQKADIAKNQADIAQNNESIEELYDFDNEVAEKIGEIHAYTEEVNKTLQDLITNSVKNTDNIDKNKADIDNNINHIYELAQQQDQHSSDIKTLKNNVEEGLLELSGHLIDQKADLTKDIKTLENNVEEGLLDLSGRLIDQKADIAKNQADIAQNQTDIQDLAAYNELQDQYAQKQTEAIDALNKASSENTQNIEDLAAYNELQDAYAKQQTEAIDALNKASSENTQNIAKNQADIANNINNIYELAQQQDQHSSDIKTLAKASAANTDRIAKNKADADASFETLTKNQNTLIEKDKEHDKLITANKTAIDENKASADTKFAATADAITKNGNAITKNAKSITDLGTKVDGFDGRVTALDTKVNAFDGRITALDSKVENGMAAQAALSGLFQPYSVGKFNATAALGGYGSKSAVAIGAGYRVNPNLAFKAGAAINTSGNKKGSYNIGVNYEF

SEQ ID NO: 31 - protein, 613 aa, Moraxella catarrhalis
MKTMKLLPLKIAVTSAMIIGLGAASTANAQSRDRSLEDIQDSISKLVQDDIDTLKQDQQKMNKYLLLNQLANTLITDELNNNVIKNTNSIEALGDEIGWLENDIADLEEGVEELTKNQNTLIEKDEEHDRLIAQNQADIQTLENNVVEELFNLSGRLIDQEADIAKNNASIEELYDFDNEVAERIGEIHAYTEEVNKTLENLITNSVKNTDNIDKNKADIDNNINHIYELAQQQDQHSSDIKTLKNNVEEGLLELSGHLIDQKADLTKDIKALESNVEEGLLDLSGRLLDQKADLTKDIKALESNVEEGLLDLSGRLLDQKADIAQNQTDIQDLAAYNELQDQYAQKQTEAIDALNKASSENTQNIEDLAAYNELQDAYAKQQTEAIDALNKASSENTQNIAKNQADIANNINNIYELAQQQDQHSSDIKTLAKASAANTNRIATAELGIAENKKDAQIAKAQANANKTAIDENKASADTKFAATADAITKNGNAITKNAKSITDLGTKVDGFDGRVTALDTKVNAFDGRITALDSKVENGMAAQAALSGLFQPYSVGKFNATAALGGYGSKSAVAIGAGYRVNPNLAFKAGAAINTSGNKKGSYNIGVNYEF

SEQ ID NO: 32 - protein, 863 aa, Moraxella catarrhalis
MNKIYKVKKNAAGHLVACSEFAKGHTKKAVLGSLLIVGILGMATTASAQKVGKATNKISGGDNNTANGTYLTIGGGDYNKTKGRYSTIGGGLFNEATNEYSTIGSGGYNKAKGRYSTIGGGGYNEATNQYSTIGGGDNNTAKGRYSTIGGGGYNEATIENSTVGGGGYNQAKGRNSTVAGGYNNEATGTDSTIAGGRKNQATGKGSFAAGIDNKANADNAVALGNKNTIEGENSVAIGSNNTVKKGQQNVFILGSNTDTTNAQNGSVLLGHNTAGKAATIVNSAEVGGLSLTGFAGASKTGNGTVSVGKKGKERQIVHVGAGEISDTSTDAVNGSQLHVLATVVAQNKADIKDLDDEVGLLGEEINSLEGEIFNNQDAIAKNQADIKTLESNVEEGLLDLSGRLLDQKADIDNNINNIYELAQQQDQHSSDIKTLKNNVEEGLLDLSGRLIDQKADLTKDIKALESNVEEGLLDLSGRLIDQKADIAKNQADIAQNQTDIQDLAAYNELQDAYAKQQTEAIDALNKASSANTDRIATAELGIAENKKDAQIAKAQANENKDGIAKNQADIQLHDKKITNLGILHSMVARAVGNNTQGVATNKADIAKNQADIANNIKNIYELAQQQDQHSSDIKTLAKVSAANTDRIAKNKAEADASFETLTKNQNTLIEQGEALVEQNKAINQELEGFAAHADVQDKQILQNQADITTNKTAIEQNINRTVANGFEIEKNKAGIATNKQELILQNDRLNRINETNNHQDQKIDQLGYALKEQGQHFNNRISAVERQTAGGIANAIAIATLPSPSRAGEHHVLFGSGYHNGQAAVSLGAAGLSDTGKSTYKIGLSWSDAGGLSGGVGGSYRWK

SEQ ID NO: 33 - protein, 630 aa, Moraxella catarrhalis
MKTMKLLPLKIAVTSAMIIGLGAASTANAQAKNDITLEDLPYLIKKIDQNELEADIGDITALEKYLALSQYGNILALEELNKALEELDEDVGWNQNDIANLEDDVETLTKNQNAFAEQGEAIKEDLQGLADFVEGQEGKILQNETSIKKNTQRNLVNGFEIEKNKDAIAKNNESIEDLYDFGHEVAESIGEIHAHNEAQNETLKGLITNSIENTNNITKNKADIQALENNVVEELFNLSGRLIDQKADIDNNINNIYELAQQQDQHSSDIKTLKKNVEEGLLELSDHIIDQKTDIAQNQANIQDLATYNELQDQYAQKQTEAIDALNKASSENTQNIEDLAAYNELQDAYAKQQTEAIDALNKASSENTQNIEDLAAYNELQDAYAKQQAEAIDALNKASSENTQNIAKNQADIANNITNLYELAQQQDKHRSDIKTLAKTSAANTDRIAKNKADDDASFETLTKNQNTLIEKDKEHDKLITANKTAIDANKASADTKFAATADAFTKNGNAITKNAKSITDLGTKVDGFDSRVTALDTKVNAFDGRITALDSKVENGMAAQAALSGLFQPYSVGKFNATAALGGYGSKSAVAIGAGYRVNPNLAFKAGAAINTSGNKKGSYNIGVNYEF

SEQ ID NO: 34 - protein, 42 aa, Moraxella catarrhalis
  MOD_RES (2): Thr or Val
  MOD_RES (7): Ser or Lys
  MOD_RES (8): Gln, Glu, Lys or Ala
  MOD_RES (9): Gly or Asn
  MOD_RES (10): Lys, Asn, Gly, His or Ser
  MOD_RES (16): Asn or His
  MOD_RES (21): Gln, Asn, Glu or Lys
  MOD_RES (23): Ser or Arg
  MOD_RES (24): Ala or Asp
  MOD_RES (25): Thr or Asp
  MOD_RES (36): His or Tyr
  MOD_RES (40): Ser, Lys or Thr
  MOD_RES (41): Thr, Ala or Val
  MOD_RES (42): Ile or Val
GXVSVGXXXXERQIVXVGAGXIXXXSTDAVNGSQLXALAXXX

SEQ ID NO: 35 - protein, 10 aa, Moraxella catarrhalis
STDAVNGSQL

SEQ ID NO: 36 - protein, 40 aa, Moraxella catarrhalis
  MOD_RES (3): Asn or Asp
  MOD_RES (9): Leu or Ile
  MOD_RES (21): Asn or His
  MOD_RES (24): Glu or Asp
LLXLSGRLXDQKADIDNNINXIYXLAQQQDQHSSDIKTLK

SEQ ID NO: 37 - protein, 11 aa, Moraxella catarrhalis
DQKADIDNNIN

SEQ ID NO: 38 - protein, 16 aa, Moraxella catarrhalis
LAQQQDQHSSDIKTLK

SEQ ID NO: 39 - protein, 24 aa, Moraxella catarrhalis
  MOD_RES (10): Asn or His
KADIDNNINXIYELAQQQDQHSSD

SEQ ID NO: 40 - protein, 29 aa, Moraxella catarrhalis
  MOD_RES (2): Lys or Gln
  MOD_RES (3): Thr or Ala
  MOD_RES (5): Lys or Glu
  MOD_RES (6): Lys, Asn or Ser
  MOD_RES (8): Val or Ile
  MOD_RES (9): Glu or Val
  MOD_RES (11): Gly or Glu
  MOD_RES (13): Leu or Phe
  MOD_RES (14): Glu or Asn
  MOD_RES (17): Asp or Gly
  MOD_RES (18): His or Arg
  MOD_RES (19): Ile or Leu
  MOD_RES (24): Thr or Ala
  MOD_RES (26): Ile or Leu
  MOD_RES (27): Ala or Thr
  MOD_RES (28): Gln or Lys
  MOD_RES (29): Asn or Asp
IXXLXXNXXEXLXXLSXXXIDQKXDXXXX

SEQ ID NO: 41 - protein, 78 aa, Moraxella catarrhalis
  MOD_RES (2): Glu or Gln
  MOD_RES (19): Ala or Thr
  MOD_RES (48): Thr or Asn
  MOD_RES (59): Lys or Gln
  MOD_RES (61): Arg or Ser
  MOD_RES (70): Thr or Ala
  MOD_RES (76): Asp or Asn
IXDLAAYNELQDAYAKQQXEAIDALNKASSENTQNIAKNQADIANNIXNIYELAQQQDXHXSDIKTLAKXSAANTXRI

SEQ ID NO: 42 - protein, 16 aa, Moraxella catarrhalis
DLAAYNELQDAYAKQQ

SEQ ID NO: 43 - protein, 28 aa, Moraxella catarrhalis
EAIDALNKASSENTQNIAKNQADIANNI

SEQ ID NO: 44 - protein, 42 aa, Moraxella catarrhalis; identical to SEQ ID NO: 34
  MOD_RES (2): Thr or Val
  MOD_RES (7): Ser or Lys
  MOD_RES (8): Gln, Glu, Lys or Ala
  MOD_RES (9): Gly or Asn
  MOD_RES (10): Lys, Asn, Gly, His or Ser
  MOD_RES (16): Asn or His
  MOD_RES (21): Gln, Asn, Glu or Lys
  MOD_RES (23): Ser or Arg
  MOD_RES (24): Ala or Asp
  MOD_RES (25): Thr or Asp
  MOD_RES (36): His or Tyr
  MOD_RES (40): Ser, Lys or Thr
  MOD_RES (41): Thr, Ala or Val
  MOD_RES (42): Ile or Val

SEQ ID NO: 45 - protein, 10 aa, Moraxella catarrhalis
STDAVNGSQL

SEQ ID NO: 46 - protein, 40 aa, Moraxella catarrhalis; identical to SEQ ID NO: 36
  MOD_RES (3): Asn or Asp
  MOD_RES (9): Leu or Ile
  MOD_RES (21): Asn or His
  MOD_RES (24): Glu or Asp

SEQ ID NO: 47 - protein, 11 aa, Moraxella catarrhalis
DQKADIDNNIN

SEQ ID NO: 48 - protein, 16 aa, Moraxella catarrhalis
LAQQQDQHSSDIKTLK

SEQ ID NO: 49 - protein, 24 aa, Moraxella catarrhalis
  MOD_RES (10): Asn or His
KADIDNNINXIYELAQQQDQHSSD

SEQ ID NO: 50 - protein, 29 aa, Moraxella catarrhalis
  MOD_RES (2): Lys or Gln
  MOD_RES (3): Thr or Ala
  MOD_RES (5): Lys or Glu
  MOD_RES (6): Lys, Asn or Ser
  MOD_RES (8): Val or Ile
  MOD_RES (9): Glu or Val
  MOD_RES (11): Gly or Glu
  MOD_RES (13): Leu or Phe
  MOD_RES (14): Glu or Asn
  MOD_RES (17): Asp or Gly
  MOD_RES (18): His or Arg
  MOD_RES (19): Ile or Leu
  MOD_RES (24): Thr or Ala
  MOD_RES (26): Ile or Leu
  MOD_RES (27): Ala or Thr
  MOD_RES (28): Gln or Lys
  MOD_RES (29): Asn or Asp
IXXLXXNXXEXLXXLSXXXIDQKXDXXXX

SEQ ID NO: 51 - protein, 78 aa, Moraxella catarrhalis; identical to SEQ ID NO: 41
  MOD_RES (2): Glu or Gln
  MOD_RES (19): Ala or Thr
  MOD_RES (48): Thr or Asn
  MOD_RES (59): Lys or Gln
  MOD_RES (61): Arg or Ser
  MOD_RES (70): Thr or Ala
  MOD_RES (76): Asp or Asn

SEQ ID NO: 52 - protein, 16 aa, Moraxella catarrhalis
DLAAYNELQDAYAKQQ

SEQ ID NO: 53 - protein, 28 aa, Moraxella catarrhalis
EAIDALNKASSENTQNIAKNQADIANNI

SEQ ID NO: 54 - DNA, 23 bp, Artificial Sequence
  Description of Artificial Sequence: Synthetic primer
caaagctgacatccaagcacttg

SEQ ID NO: 55 - DNA, 30 bp, Artificial Sequence
  Description of Artificial Sequence: Synthetic primer
gcgtctgcggatccagtaggcaaggcaacc

SEQ ID NO: 56 - DNA, 30 bp, Artificial Sequence; identical to SEQ ID NO: 55
  Description of Artificial Sequence: Synthetic primer

SEQ ID NO: 57 - DNA, 30 bp, Artificial Sequence; identical to SEQ ID NO: 55
  Description of Artificial Sequence: Synthetic primer

SEQ ID NO: 58 - DNA, 30 bp, Artificial Sequence; identical to SEQ ID NO: 55
  Description of Artificial Sequence: Synthetic primer

SEQ ID NO: 59 - DNA, 36 bp, Artificial Sequence
  Description of Artificial Sequence: Synthetic primer
ggatttgcaggtgcatcggatcctggtaatggtact

SEQ ID NO: 60 - DNA, 30 bp, Artificial Sequence
  Description of Artificial Sequence: Synthetic primer
catagctctgatatggatccacttaaaaac

SEQ ID NO: 61 - DNA, 30 bp, Artificial Sequence
  Description of Artificial Sequence: Synthetic primer
gccaaagcacaagcggatccaaataaagac

SEQ ID NO: 62 - DNA, 30 bp, Artificial Sequence
  Description of Artificial Sequence: Synthetic primer
gttgagcaaaaggatcccatcaatcaagag

SEQ ID NO: 63 - DNA, 36 bp, Artificial Sequence
  Description of Artificial Sequence: Synthetic primer
cgaatgcggatcctaaaaatgatataactttagagg

SEQ ID NO: 64 - DNA, 36 bp, Artificial Sequence; identical to SEQ ID NO: 63
  Description of Artificial Sequence: Synthetic primer

SEQ ID NO: 65 - DNA, 32 bp, Artificial Sequence
  Description of Artificial Sequence: Synthetic primer
gatattgcggatccggaagatgatgttgaaac

SEQ ID NO: 66 - DNA, 32 bp, Artificial Sequence; identical to SEQ ID NO: 65
  Description of Artificial Sequence: Synthetic primer

SEQ ID NO: 67 - DNA, 30 bp, Artificial Sequence
  Description of Artificial Sequence: Synthetic primer
gagattgagaaggatccagatgctattgct

SEQ ID NO: 68 - DNA, 30 bp, Artificial Sequence
  Description of Artificial Sequence: Synthetic primer
gctcaaaaccaagcggatccccaagatctg

SEQ ID NO: 69 - DNA, 30 bp, Artificial Sequence
  Description of Artificial Sequence: Synthetic primer
gcaagtgctgcggatcctgatcgtattgct

SEQ ID NO: 70 - DNA, 29 bp, Artificial Sequence
  Description of Artificial Sequence: Synthetic primer
ccctgaagctttagtgcataacctaattg

SEQ ID NO: 71 - DNA, 28 bp, Artificial Sequence
  Description of Artificial Sequence: Synthetic primer
ttgagcaagcttagcttggtttttagcg

SEQ ID NO: 72 - DNA, 24 bp, Artificial Sequence
  Description of Artificial Sequence: Synthetic primer
acctgtggcaagcttcttcctgcc

SEQ ID NO: 73 - DNA, 33 bp, Artificial Sequence
  Description of Artificial Sequence: Synthetic primer
ggtgtcactaagcttacctgcaccaacatgaac

SEQ ID NO: 74 - DNA, 30 bp, Artificial Sequence
  Description of Artificial Sequence: Synthetic primer
gtcttttgtaagatcaagcttttgatcaat

SEQ ID NO: 75 - DNA, 26 bp, Artificial Sequence
  Description of Artificial Sequence: Synthetic primer
catgctgagaagcttacctagattgg

SEQ ID NO: 76 - DNA, 33 bp, Artificial Sequence
  Description of Artificial Sequence: Synthetic primer
ggtcttattggtagtaagcttagcttggttttg

SEQ ID NO: 77 - DNA, 29 bp, Artificial Sequence
  Description of Artificial Sequence: Synthetic primer
ccctgaagctttagtgcataacctaattg

SEQ ID NO: 78 - DNA, 28 bp, Artificial Sequence
  Description of Artificial Sequence: Synthetic primer
cattaagcttggtgtctaatgcagttac

SEQ ID NO: 79 - DNA, 36 bp, Artificial Sequence
  Description of Artificial Sequence: Synthetic primer
ctcatgaccaaaatcaagcttatcttcgatagactc

SEQ ID NO: 80 - DNA, 37 bp, Artificial Sequence
  Description of Artificial Sequence: Synthetic primer
gatcaataagcttaccgcttagattgaatagttcttc

SEQ ID NO: 81 - DNA, 33 bp, Artificial Sequence
  Description of Artificial Sequence: Synthetic primer
gtcaatcgcttcaagcttcttttgagcatactg

SEQ ID NO: 82 - DNA, 33 bp, Artificial Sequence; identical to SEQ ID NO: 81
  Description of Artificial Sequence: Synthetic primer

SEQ ID NO: 83 - DNA, 33 bp, Artificial Sequence
  Description of Artificial Sequence: Synthetic primer
ggtgagcgtttcaagctttgcatcagcatcggc

SEQ ID NO: 84 - DNA, 28 bp, Artificial Sequence
  Description of Artificial Sequence: Synthetic primer
cattaagcttggtgtctaatgcagttac

SEQ ID NO: 85 - protein, 23 aa, Moraxella catarrhalis
NNINNIYELAQQQDQHSSDIKTL

SEQ ID NO: 86 - protein, 7 aa, Moraxella catarrhalis
NNINNIY